European Patent Application EP 4 570 907 A1, published June 18, 2025. Title: Methods for selecting subject-derived neoantigens. Applicant: Sapporo Medical University. Application JP 2022-126148, filed August 8, 2022. The sequence listing filed with the application follows.

SEQUENCE LISTING (11 sequences)

SEQ ID NO: 1 - protein, 9 aa, Mus musculus
KYLSVQSQL

SEQ ID NO: 2 - protein, 9 aa, Mus musculus
KYSNASEAI

SEQ ID NO: 3 - protein, 9 aa, Mus musculus
KGPKRDEQC

SEQ ID NO: 4 - protein, 8 aa, Mus musculus
QPVSSLRF

SEQ ID NO: 5 - protein, 9 aa, Mus musculus
ARPTVVSHL

SEQ ID NO: 6 - protein, 10 aa, Mus musculus
HRQERRERPY

SEQ ID NO: 7 - protein, 9 aa, Homo sapiens
RYLAVAAVF

SEQ ID NO: 8 - protein, 9 aa, Homo sapiens
KLNPQRFEV

SEQ ID NO: 9 - protein, 9 aa, Human immunodeficiency virus
RYLRDQQLL

SEQ ID NO: 10 - protein, 9 aa, Human immunodeficiency virus
SLYNTVATL

SEQ ID NO: 11 - protein, 15 aa, Homo sapiens
KGEIAASIVTHMRPY